European Patent Application EP 4 169 949 A1, published April 26, 2023. Title: ANTI-CD38 ANTIBODY AND USE THEREOF. Applicant: JIANGSU KANION PHARMACEUTICAL CO.,LTD. The sequence listing filed with the application follows.

SEQUENCE LISTING (43 sequences)

SEQ ID NO: 1 - protein, 300 aa, Homo sapiens
MANCEFSPVSGDKPCCRLSRRAQLCLGVSILVLILVVVLAVVVPRWRQQWSGPGTTKRFPETVLARCVKYTEIHPEMRHVDCQSVWDAFKGAFISKHPCNITEEDYQPLMKLGTQTVPCNKILLWSRIKDLAHQFTQVQRDMFTLEDTLLGYLADDLTWCGEFNTSKINYQSCPDWRKDCSNNPVSVFWKTVSRRFAEAACDVVHVMLNGSRSKIFDKNSTFGSVEVHNLQPEKVQTLEAWVIHGGREDSRDLCQDPTIKELESIISKRNIQFSCKNIYRPDKFLQCVKNPEDSSCTSEI

SEQ ID NO: 2 - DNA, 780 bp, Artifical Sequence
  scFv418 nucleic acid sequence
caatctgccctgactcagcctgcctccgtgtctgggtctcctggacagtcgatcaccatctcctgcactggaaccagcagtgacgttggtggttataactatgtctcctggtaccaacagcacccaggcaaagcccccaaactcgtaatttatgagggcactcagcggccctcaggggtttctagtcgcttctctggctccaagtctggcaacacggcctccctgacaatctctgggctccaggctgaggacgaggctgattattactgcagctcatacacaagcagcagtttttatgtcttcggaactgggaccaagctgaccgtcctagtcgacggtggaggtggcagtggaggtggcggttctggcggtggaggttctgctagccaggtacagctgcagcagtcaggtccaggactggtgaagccctcgcagaccctctcactcacctgtgccatctccgggggcagtgtctctagcaacagtgctgcttggaactggatcaggcagtccccatcgagaggccttgagtggctgggaaggacatactacaggtccaagtggtataatgattatgcagtatctgtgaaaagtcgaataaccatcaacccagacacatccaagaaccagttctccctgcagctgaactctgtgactcccgaggacacggctgtgtattactgtgcaagagatgcgctagcagcagctggtacatatggttactactactactacggtatggacgtctggggccaagggacaatggtcaccgtctcttca

SEQ ID NO: 3 - protein, 260 aa, Artifical Sequence
  scFv418 amino acid sequence
QSALTQPASVSGSPGQSITISCTGTSSDVGGYNYVSWYQQHPGKAPKLVIYEGTQRPSGVSSRFSGSKSGNTASLTISGLQAEDEADYYCSSYTSSSFYVFGTGTKLTVLVDGGGGSGGGGSGGGGSASQVQLQQSGPGLVKPSQTLSLTCAISGGSVSSNSAAWNWIRQSPSRGLEWLGRTYYRSKWYNDYAVSVKSRITINPDTSKNQFSLQLNSVTPEDTAVYYCARDALAAAGTYGYYYYYGMDVWGQGTMVTVSS

SEQ ID NO: 4 - DNA, 393 bp, Artifical Sequence
  scFv418 VH nucleic acid sequence
caggtacagctgcagcagtcaggtccaggactggtgaagccctcgcagaccctctcactcacctgtgccatctccgggggcagtgtctctagcaacagtgctgcttggaactggatcaggcagtccccatcgagaggccttgagtggctgggaaggacatactacaggtccaagtggtataatgattatgcagtatctgtgaaaagtcgaataaccatcaacccagacacatccaagaaccagttctccctgcagctgaactctgtgactcccgaggacacggctgtgtattactgtgcaagagatgcgctagcagcagctggtacatatggttactactactactacggtatggacgtctggggccaagggacaatggtcaccgtctcttca

SEQ ID NO: 5 - protein, 131 aa, Artifical Sequence
  scFv418 VH amino acid sequence
QVQLQQSGPGLVKPSQTLSLTCAISGGSVSSNSAAWNWIRQSPSRGLEWLGRTYYRSKWYNDYAVSVKSRITINPDTSKNQFSLQLNSVTPEDTAVYYCARDALAAAGTYGYYYYYGMDVWGQGTMVTVSS

SEQ ID NO: 6 - DNA, 75 bp, Artifical Sequence
  scFv418 VH frame region 1 (FR1) nucleic acid sequence
caggtacagctgcagcagtcaggtccaggactggtgaagccctcgcagaccctctcactcacctgtgccatctcc

SEQ ID NO: 7 - protein, 25 aa, Artifical Sequence
  scFv418 VH frame region 1 (FR1) amino acid sequence
QVQLQQSGPGLVKPSQTLSLTCAIS

SEQ ID NO: 8 - DNA, 30 bp, Artifical Sequence
  scFv418 VH CDR1 nucleic acid sequence
gggggcagtgtctctagcaacagtgctgct

SEQ ID NO: 9 - protein, 10 aa, Artifical Sequence
  scFv418 VH CDR1 amino acid sequence
GGSVSSNSAA

SEQ ID NO: 10 - DNA, 51 bp, Artifical Sequence
  scFv418 VH frame region 2 (FR2) nucleic acid sequence
tggaactggatcaggcagtccccatcgagaggccttgagtggctgggaagg

SEQ ID NO: 11 - protein, 17 aa, Artifical Sequence
  scFv418 VH frame region 2 (FR2) amino acid sequence
WNWIRQSPSRGLEWLGR

SEQ ID NO: 12 - DNA, 27 bp, Artifical Sequence
  scFv418 VH CDR2 nucleic acid sequence
acatactacaggtccaagtggtataat

SEQ ID NO: 13 - protein, 9 aa, Artifical Sequence
  scFv418 VH CDR2 amino acid sequence
TYYRSKWYN

SEQ ID NO: 14 - DNA, 114 bp, Artifical Sequence
  scFv418 VH frame region 3 (FR3) nucleic acid sequence
gattatgcagtatctgtgaaaagtcgaataaccatcaacccagacacatccaagaaccagttctccctgcagctgaactctgtgactcccgaggacacggctgtgtattactgt

SEQ ID NO: 15 - protein, 38 aa, Artifical Sequence
  scFv418 VH frame region 3 (FR3) amino acid sequence
DYAVSVKSRITINPDTSKNQFSLQLNSVTPEDTAVYYC

SEQ ID NO: 16 - DNA, 63 bp, Artifical Sequence
  scFv418 VH CDR3 nucleic acid sequence
gcaagagatgcgctagcagcagctggtacatatggttactactactactacggtatggacgtc

SEQ ID NO: 17 - protein, 21 aa, Artifical Sequence
  scFv418 VH CDR3 amino acid sequence
ARDALAAAGTYGYYYYYGMDV

SEQ ID NO: 18 - DNA, 33 bp, Artifical Sequence
  scFv418 VH frame region 4 (FR4) nucleic acid sequence
tggggccaagggacaatggtcaccgtctcttca

SEQ ID NO: 19 - protein, 11 aa, Artifical Sequence
  scFv418 VH frame region 4 (FR4) amino acid sequence
WGQGTMVTVSS

SEQ ID NO: 20 - DNA, 330 bp, Artifical Sequence
  scFv418 VL nucleic acid sequence
caatctgccctgactcagcctgcctccgtgtctgggtctcctggacagtcgatcaccatctcctgcactggaaccagcagtgacgttggtggttataactatgtctcctggtaccaacagcacccaggcaaagcccccaaactcgtaatttatgagggcactcagcggccctcaggggtttctagtcgcttctctggctccaagtctggcaacacggcctccctgacaatctctgggctccaggctgaggacgaggctgattattactgcagctcatacacaagcagcagtttttatgtcttcggaactgggaccaagctgaccgtccta

SEQ ID NO: 21 - protein, 110 aa, Artifical Sequence
  scFv418 VL amino acid sequence
QSALTQPASVSGSPGQSITISCTGTSSDVGGYNYVSWYQQHPGKAPKLVIYEGTQRPSGVSSRFSGSKSGNTASLTISGLQAEDEADYYCSSYTSSSFYVFGTGTKLTVL

SEQ ID NO: 22 - DNA, 75 bp, Artifical Sequence
  scFv418 VL frame region (FR1) nucleic acid sequence
caatctgccctgactcagcctgcctccgtgtctgggtctcctggacagtcgatcaccatctcctgcactggaacc

SEQ ID NO: 23 - protein, 25 aa, Artifical Sequence
  scFv418 VL frame region (FR1) amino acid sequence
QSALTQPASVSGSPGQSITISCTGT

SEQ ID NO: 24 - DNA, 27 bp, Artifical Sequence
  scFv418 VL CDR1 nucleic acid sequence
agcagtgacgttggtggttataactat

SEQ ID NO: 25 - protein, 9 aa, Artifical Sequence
  scFv418 VL CDR1 amino acid sequence
SSDVGGYNY

SEQ ID NO: 26 - DNA, 51 bp, Artifical Sequence
  scFv418 VL frame region 2 (FR2) nucleic acid sequence
gtctcctggtaccaacagcacccaggcaaagcccccaaactcgtaatttat

SEQ ID NO: 27 - protein, 17 aa, Artifical Sequence
  scFv418 VL frame region 2 (FR2) amino acid sequence
VSWYQQHPGKAPKLVIY

SEQ ID NO: 28 - DNA, 9 bp, Artifical Sequence
  scFv418 VL CDR2 nucleic acid sequence
gagggcact

SEQ ID NO: 29 - protein, 3 aa, Artifical Sequence
  scFv418 VL CDR2 amino acid sequence
EGT

SEQ ID NO: 30 - DNA, 108 bp, Artifical Sequence
  scFv418 VL frame region 3 (FR3) nucleic acid sequence
cagcggccctcaggggtttctagtcgcttctctggctccaagtctggcaacacggcctccctgacaatctctgggctccaggctgaggacgaggctgattattactgc

SEQ ID NO: 31 - protein, 36 aa, Artifical Sequence
  scFv418 VL frame region 3 (FR3) amino acid sequence
QRPSGVSSRFSGSKSGNTASLTISGLQAEDEADYYC

SEQ ID NO: 32 - DNA, 30 bp, Artifical Sequence
  scFv418 VL CDR3 nucleic acid sequence
agctcatacacaagcagcagtttttatgtc

SEQ ID NO: 33 - protein, 10 aa, Artifical Sequence
  scFv418 VL CDR3 amino acid sequence
SSYTSSSFYV

SEQ ID NO: 34 - DNA, 30 bp, Artifical Sequence
  scFv418 VL frame region 4 (FR4) nucleic acid sequence
ttcggaactgggaccaagctgaccgtccta

SEQ ID NO: 35 - protein, 10 aa, Artifical Sequence
  scFv418 VL frame region 4 (FR4) amino acid sequence
FGTGTKLTVL

SEQ ID NO: 36 - DNA, 1386 bp, Artifical Sequence
  IgG418 heavy chain nucleic acid sequence
caggtacagctgcagcagtcaggtccaggactggtgaagccctcgcagaccctctcactcacctgtgccatctccgggggcagtgtctctagcaacagtgctgcttggaactggatcaggcagtccccatcgagaggccttgagtggctgggaaggacatactacaggtccaagtggtataatgattatgcagtatctgtgaaaagtcgaataaccatcaacccagacacatccaagaaccagttctccctgcagctgaactctgtgactcccgaggacacggctgtgtattactgtgcaagagatgcgctagcagcagctggtacatatggttactactactactacggtatggacgtctggggccaagggacaatggtcaccgtctcttcagcctccactaagggcccatccgtgttcccactggcaccctctagtaagagcacatctgggggtactgccgctctgggatgtctggtgaaggattacttcccagagccagtcaccgtgtcctggaacagcggggccctgacttccggtgtccatacctttccagctgtgctgcagtcatccggcctgtacagcctgagctctgtggtcaccgtccccagttcatccctgggaacacagacttatatctgcaacgtgaatcacaagccatccaatacaaaagtcgacaagaaagtggaacccaagagctgtgataaaacccatacatgccccccttgtcctgctccagagctgctgggaggaccatccgtgttcctgtttccacccaagcctaaagacactctgatgatttctcgaacccccgaagtcacatgcgtggtcgtggacgtgtcccacgaggatcctgaagtcaagttcaactggtacgtggatggcgtcgaggtgcataatgccaagacaaaaccacgagaggaacagtacaacagtacctatcgtgtcgtgtcagtcctgacagtgctgcaccaggactggctgaacgggaaggaatataagtgcaaagtgagcaataaggcactgcccgcccctatcgagaaaacaatttctaaggctaaaggacagcctagggaaccacaggtgtacactctgcctccatcacgggacgagctgacaaagaaccaggtcagtctgacttgtctggtgaaagggttctatccttctgatatcgccgtggagtgggaaagtaatggtcagccagagaacaattacaagaccacaccccctgtcctggactctgatgggagtttctttctgtattccaagctgaccgtggataaaagccggtggcagcagggtaatgtctttagttgttcagtgatgcacgaggcactgcacaatcactacacccagaaatcactgtcactgtcaccaggtaaatga

SEQ ID NO: 37 - protein, 461 aa, Artifical Sequence
  IgG418 heavy chain amino acid sequence
QVQLQQSGPGLVKPSQTLSLTCAISGGSVSSNSAAWNWIRQSPSRGLEWLGRTYYRSKWYNDYAVSVKSRITINPDTSKNQFSLQLNSVTPEDTAVYYCARDALAAAGTYGYYYYYGMDVWGQGTMVTVSSASTKGPSVFPLAPSSKSTSGGTAALGCLVKDYFPEPVTVSWNSGALTSGVHTFPAVLQSSGLYSLSSVVTVPSSSLGTQTYICNVNHKPSNTKVDKKVEPKSCDKTHTCPPCPAPELLGGPSVFLFPPKPKDTLMISRTPEVTCVVVDVSHEDPEVKFNWYVDGVEVHNAKTKPREEQYNSTYRVVSVLTVLHQDWLNGKEYKCKVSNKALPAPIEKTISKAKGQPREPQVYTLPPSRDELTKNQVSLTCLVKGFYPSDIAVEWESNGQPENNYKTTPPVLDSDGSFFLYSKLTVDKSRWQQGNVFSCSVMHEALHNHYTQKSLSLSPGK

SEQ ID NO: 38 - DNA, 60 bp, Artifical Sequence
  IgG418 heavy chain signal peptide nucleic acid sequence
atgtctgtctccttcctcatcttcctgcccgtgctgggcctcccatggggtgtcctgtca

SEQ ID NO: 39 - protein, 20 aa, Artifical Sequence
  IgG418 heavy chain signal peptide amino acid sequence
MSVSFLIFLPVLGLPWGVLS

SEQ ID NO: 40 - DNA, 651 bp, Artifical Sequence
  IgG418 light chain nucleic acid sequence
caatctgccctgactcagcctgcctccgtgtctgggtctcctggacagtcgatcaccatctcctgcactggaaccagcagtgacgttggtggttataactatgtctcctggtaccaacagcacccaggcaaagcccccaaactcgtaatttatgagggcactcagcggccctcaggggtttctagtcgcttctctggctccaagtctggcaacacggcctccctgacaatctctgggctccaggctgaggacgaggctgattattactgcagctcatacacaagcagcagtttttatgtcttcggaactgggaccaagctgaccgtcctaggtcagcctaaggctgctcctagcgtgaccctgttccctcccagcagcgaggagctgcaggcaaacaaagccaccctggtgtgcctgatctccgacttttaccctggcgccgtgacagtggcctggaaggctgacagcagcccagtgaaagccggagtggagaccaccaccccctccaagcagtccaacaacaagtacgccgcatcctcctacctgagcctgacccccgagcagtggaagtcccacaggtcctactcctgccaggtgacccacgagggctctaccgtggaaaagaccgtggcccccaccgagtgctcctga

SEQ ID NO: 41 - protein, 216 aa, Artifical Sequence
  IgG418 light chain amino acid sequence
QSALTQPASVSGSPGQSITISCTGTSSDVGGYNYVSWYQQHPGKAPKLVIYEGTQRPSGVSSRFSGSKSGNTASLTISGLQAEDEADYYCSSYTSSSFYVFGTGTKLTVLGQPKAAPSVTLFPPSSEELQANKATLVCLISDFYPGAVTVAWKADSSPVKAGVETTTPSKQSNNKYAASSYLSLTPEQWKSHRSYSCQVTHEGSTVEKTVAPTECS

SEQ ID NO: 42 - DNA, 57 bp, Artifical Sequence
  IgG418 light chain signal peptide nucleic acid sequence
atggcctgggctctgctgctcctcaccctcctcactcagggcacagggtcctgggcc

SEQ ID NO: 43 - protein, 19 aa, Artifical Sequence
  IgG418 light chain signal peptide amino acid sequence
MAWALLLLTLLTQGTGSWA